European Patent Application EP 4 159 748 A1, published April 5, 2023. Title: INTERLEUKIN 29 MUTANT PROTEIN. Applicant: SCIWIND BIOSCIENCES CO., LTD. Application PCT/CN2021/075907. The sequence listing filed with the application follows.

SEQUENCE LISTING (18 sequences)

SEQ ID NO: 1 - protein, 175 aa, Artificial Sequence
  Artificial
KPTTTGKGCHIGRFKSLSPQELASFKKARDALEESLKLKNWSCSSPVFPGNWDLRLLQVRERPVALEAELALTLKVLEAAAGPALEDVLDQPLHTLHHILSQLQACIQPQPTAGPRPRGRLHHWLHRLQEAPKKESAGCLEASVTFNLFRLLTRDLKYVADGNLCLRTSTHPEST

SEQ ID NO: 2 - protein, 181 aa, Artificial Sequence
  Artificial
GPVPTSKPTTTGKGCHIGRFKSLSPQELASFKKARDALEESLKLKNWSCSSPVFPGNWDLRLLQVRERPVALEAELALTLKVLEAAAGPALEDVLDQPLHTLHHILSQLQACIQPQPTAGPRPRGRLHHWLHRLQEAPKKESAGCLEASVTFNLFRLLTRDLKYVADGNLCLRTSTHPEST

SEQ ID NO: 3 - protein, 200 aa, Artificial Sequence
  Artificial
MAAAWTVVLVTLVLGLAVAGPVPTSKPTTTGKGCHIGRFKSLSPQELASFKKARDALEESLKLKNWSCSSPVFPGNWDLRLLQVRERPVALEAELALTLKVLEAAAGPALEDVLDQPLHTLHHILSQLQACIQPQPTAGPRPRGRLHHWLHRLQEAPKKESAGCLEASVTFNLFRLLTRDLKYVADGNLCLRTSTHPEST

SEQ ID NO: 4 - protein, 176 aa, Artificial Sequence
  Artificial
MKPTTTGKGCHIGRFKSLSPQELASFKKARDALEESLKLKNWSCSSPVFPGNWDLRLLQVRERPVALEAELALTLKVLEAAAGPALEDVLDQPLHTLHHILSQLQACIQPQPTAGPRPRGRLHHWLHRLQEAPKKESAGCLEASVTFNLFRLLTRDLKYVAEGNLCLRTSTHPEST

SEQ ID NO: 5 - protein, 176 aa, Artificial Sequence
  Artificial
MKPTTTGKGCHIGRFKSLSPQELASFKKARDALEESLKLKNWSCSSPVFPGNWDLRLLQVRERPVALEAELALTLKVLEAAAGPALEDVLDQPLHTLHHILSQLQACIQPQPTAGPRPRGRLHHWLHRLQEAPKKESAGCLEASVTFNLFRLLTRDLKYVAEGNLSLRTSTHPEST

SEQ ID NO: 6 - protein, 176 aa, Artificial Sequence
  Artificial
MKPTTTGKGCHIGRFKSLSPQELASFKKARDALEESLKLKNWSCSSPVFPGNWDLRLLQVRERPVALEAELALTLKVLEAAAGPALEDVLDQPLHTLHHILSQLQACIQPQPTAGPRPRGRLHHWLHRLQEAPKKESAGCLEASVTFNLFRLLTRDLKYVASGNLCLRTSTHPEST

SEQ ID NO: 7 - protein, 176 aa, Artificial Sequence
  Artificial
MKPTTTGKGCHIGRFKSLSPQELASFKKARDALEESLKLKNWSCSSPVFPGNWDLRLLQVRERPVALEAELALTLKVLEAAAGPALEDVLDQPLHTLHHILSQLQACIQPQPTAGPRPRGRLHHWLHRLQEAPKKESAGCLEASVTFNLFRLLTRDLKYVASGNLSLRTSTHPEST

SEQ ID NO: 8 - protein, 176 aa, Artificial Sequence
  Artificial
MKPTTTGKGCHIGRFKSLSPQELASFKKARDALEESLKLKNWSCSSPVFPGNWDLRLLQVRERPVALEAELALTLKVLEAAAGPALEDVLDQPLHTLHHILSQLQACIQPQPTAGPRPRGRLHHWLHRLQEAPKKESAGCLEASVTFNLFRLLTRDLKYVADANLCLRTSTHPEST

SEQ ID NO: 9 - protein, 176 aa, Artificial Sequence
  Artificial
MKPTTTGKGCHIGRFKSLSPQELASFKKARDALEESLKLKNWSCSSPVFPGNWDLRLLQVRERPVALEAELALTLKVLEAAAGPALEDVLDQPLHTLHHILSQLQACIQPQPTAGPRPRGRLHHWLHRLQEAPKKESAGCLEASVTFNLFRLLTRDLKYVADANLSLRTSTHPEST

SEQ ID NO: 10 - protein, 176 aa, Artificial Sequence
  Artificial
MKPTTTGKGCHIGRFKSLSPQELASFKKARDALEESLKLKNWSCSSPVFPGNWDLRLLQVRERPVALEAELALTLKVLEAAAGPALEDVLDQPLHTLHHILSQLQACIQPQPTAGPRPRGRLHHWLHRLQEAPKKESAGCLEASVTFNLFRLLTRDLKYVADGNLSLRTSTHPEST

SEQ ID NO: 11 - DNA, 528 bp, Artificial Sequence
  Artificial
atgaaaccgaccacgaccggcaaaggctgccatattggtcgctttaagtcgctgtcgccgcaggaactggcgagcttcaagaaagcccgtgatgccctggaggaatcgctgaaactgaagaactggagctgtagctcgccggtgttcccgggcaactgggatctgcgtctgctgcaggttcgcgaacgtccggttgcgctggaagcggaactggcgctgaccctgaaagtgctggaagcggcagcgggtccggcgctggaagatgttctggatcagccgctgcacaccctgcatcatattctgtcgcagctgcaggcgtgcattcaaccgcagccgaccgcgggcccgcgtccgcgcggccgtctgcatcactggctgcaccgtctgcaggaagccccgaagaaagagtcggcgggctgtctggaagcgtcggtgaccttcaatctgttccgtctgctgacccgtgatctgaaatacgttgcggaaggcaatctgtctctgcgtacctcgacccacccggaatcgacc

SEQ ID NO: 12 - DNA, 537 bp, Artificial Sequence
  Artificial
atgaaaccgaccacgaccggcaaaggctgccatattggtcgctttaagtcgctgtcgccgcaggaactggcgagcttcaagaaagcccgtgatgccctggaggaatcgctgaaactgaagaactggagctgtagctcgccggtgttcccgggcaactgggatctgcgtctgctgcaggttcgcgaacgtccggttgcgctggaagcggaactggcgctgaccctgaaagtgctggaagcggcagcgggtccggcgctggaagatgttctggatcagccgctgcacaccctgcatcatattctgtcgcagctgcaggcgtgcattcaaccgcagccgaccgcgggcccgcgtccgcgcggccgtctgcatcactggctgcaccgtctgcaggaagccccgaagaaagagtcggcgggctgtctggaagcgtcggtgaccttcaatctgttccgtctgctgacccgtgatctgaaatacgttgcgagcggcaatctgtctctgcgtacctcgacccacccggaatcgacctaataataa

SEQ ID NO: 13 - DNA, 537 bp, Artificial Sequence
  Artificial
atgaaaccgaccacgaccggcaaaggctgccatattggtcgctttaagtcgctgtcgccgcaggaactggcgagcttcaagaaagcccgtgatgccctggaggaatcgctgaaactgaagaactggagctgtagctcgccggtgttcccgggcaactgggatctgcgtctgctgcaggttcgcgaacgtccggttgcgctggaagcggaactggcgctgaccctgaaagtgctggaagcggcagcgggtccggcgctggaagatgttctggatcagccgctgcacaccctgcatcatattctgtcgcagctgcaggcgtgcattcaaccgcagccgaccgcgggcccgcgtccgcgcggccgtctgcatcactggctgcaccgtctgcaggaagccccgaagaaagagtcggcgggctgtctggaagcgtcggtgaccttcaatctgttccgtctgctgacccgtgatctgaaatacgttgcggacgcgaatctgtctctgcgtacctcgacccacccggaatcgacctaataataa

SEQ ID NO: 14 - DNA, 528 bp, Artificial Sequence
  Artificial
atgaaaccgaccacgaccggcaaaggctgccatattggtcgctttaagtcgctgtcgccgcaggaactggcgagcttcaagaaagcccgtgatgccctggaggaatcgctgaaactgaagaactggagctgtagctcgccggtgttcccgggcaactgggatctgcgtctgctgcaggttcgcgaacgtccggttgcgctggaagcggaactggcgctgaccctgaaagtgctggaagcggcagcgggtccggcgctggaagatgttctggatcagccgctgcacaccctgcatcatattctgtcgcagctgcaggcgtgcattcaaccgcagccgaccgcgggcccgcgtccgcgcggccgtctgcatcactggctgcaccgtctgcaggaagccccgaagaaagagtcggcgggctgtctggaagcgtcggtgaccttcaatctgttccgtctgctgacccgtgatctgaaatacgttgcggaaggcaatctgtgtctgcgtacctcgacccacccggaatcgacc

SEQ ID NO: 15 - DNA, 537 bp, Artificial Sequence
  Artificial
atgaaaccgaccacgaccggcaaaggctgccatattggtcgctttaagtcgctgtcgccgcaggaactggcgagcttcaagaaagcccgtgatgccctggaggaatcgctgaaactgaagaactggagctgtagctcgccggtgttcccgggcaactgggatctgcgtctgctgcaggttcgcgaacgtccggttgcgctggaagcggaactggcgctgaccctgaaagtgctggaagcggcagcgggtccggcgctggaagatgttctggatcagccgctgcacaccctgcatcatattctgtcgcagctgcaggcgtgcattcaaccgcagccgaccgcgggcccgcgtccgcgcggccgtctgcatcactggctgcaccgtctgcaggaagccccgaagaaagagtcggcgggctgtctggaagcgtcggtgaccttcaatctgttccgtctgctgacccgtgatctgaaatacgttgcgagcggcaatctgtgtctgcgtacctcgacccacccggaatcgacctaataataa

SEQ ID NO: 16 - DNA, 537 bp, Artificial Sequence
  Artificial
atgaaaccgaccacgaccggcaaaggctgccatattggtcgctttaagtcgctgtcgccgcaggaactggcgagcttcaagaaagcccgtgatgccctggaggaatcgctgaaactgaagaactggagctgtagctcgccggtgttcccgggcaactgggatctgcgtctgctgcaggttcgcgaacgtccggttgcgctggaagcggaactggcgctgaccctgaaagtgctggaagcggcagcgggtccggcgctggaagatgttctggatcagccgctgcacaccctgcatcatattctgtcgcagctgcaggcgtgcattcaaccgcagccgaccgcgggcccgcgtccgcgcggccgtctgcatcactggctgcaccgtctgcaggaagccccgaagaaagagtcggcgggctgtctggaagcgtcggtgaccttcaatctgttccgtctgctgacccgtgatctgaaatacgttgcggacgcgaatctgtgtctgcgtacctcgacccacccggaatcgacctaataataa

SEQ ID NO: 17 - DNA, 537 bp, Artificial Sequence
  Artificial
atgaaaccgaccacgaccggcaaaggctgccatattggtcgctttaagtcgctgtcgccgcaggaactggcgagcttcaagaaagcccgtgatgccctggaggaatcgctgaaactgaagaactggagctgtagctcgccggtgttcccgggcaactgggatctgcgtctgctgcaggttcgcgaacgtccggttgcgctggaagcggaactggcgctgaccctgaaagtgctggaagcggcagcgggtccggcgctggaagatgttctggatcagccgctgcacaccctgcatcatattctgtcgcagctgcaggcgtgcattcaaccgcagccgaccgcgggcccgcgtccgcgcggccgtctgcatcactggctgcaccgtctgcaggaagccccgaagaaagagtcggcgggctgtctggaagcgtcggtgaccttcaatctgttccgtctgctgacccgtgatctgaaatacgttgcggacggcaatctgtctctgcgtacctcgacccacccggaatcgacctaataataa

SEQ ID NO: 18 - DNA, 534 bp, Artificial Sequence
  Artificial
aaaccgaccacgaccggcaaaggctgccatattggtcgctttaagtcgctgtcgccgcaggaactggcgagcttcaagaaagcccgtgatgccctggaggaatcgctgaaactgaagaactggagctgtagctcgccggtgttcccgggcaactgggatctgcgtctgctgcaggttcgcgaacgtccggttgcgctggaagcggaactggcgctgaccctgaaagtgctggaagcggcagcgggtccggcgctggaagatgttctggatcagccgctgcacaccctgcatcatattctgtcgcagctgcaggcgtgcattcaaccgcagccgaccgcgggcccgcgtccgcgcggccgtctgcatcactggctgcaccgtctgcaggaagccccgaagaaagagtcggcgggctgtctggaagcgtcggtgaccttcaatctgttccgtctgctgacccgtgatctgaaatacgttgcggacggcaatctgtgtctgcgtacctcgacccacccggaatcgacctaataataa